European Patent Application EP 4 332 118 A1, published March 6, 2024. Title: Novel Anti-CD5 Chimeric Antigen Receptor and Immune Cells Expressing the Same. Applicant: Korea Research Institute of Bioscience & Biotechnology. The sequence listing filed with the application follows.

SEQUENCE LISTING (48 sequences)

SEQ ID NO: 1 - protein, 22 aa, Artificial Sequence
  Leader sequence
MKYLLPTAAAGLLLLAAQPAMA

SEQ ID NO: 2 - protein, 5 aa, Artificial Sequence
  CD5 #1 CDR1-VH
DYGMH

SEQ ID NO: 3 - protein, 17 aa, Artificial Sequence
  CD5 #1 CDR2-VH
AISGSGSSTHYADSVKG

SEQ ID NO: 4 - protein, 12 aa, Artificial Sequence
  CD5 #1 CDR3-VH
GSSSVYSEAMDL

SEQ ID NO: 5 - protein, 119 aa, Artificial Sequence
  CD5 #1 Variable Heavy Chain
EVQLVESGGGLVQPGGSLRLSCAASGFTFSDYGMHWVRQAPGKGLEWVSAISGSGSSTHYADSVKGRFTISRDNSKNTLYLQMNSLRAEDTAVYYCAKGSSSVYSEAMDLWGQGTLVTV

SEQ ID NO: 6 - protein, 11 aa, Artificial Sequence
  CD5 #1 CDR1-VL
RASQDISSYLN

SEQ ID NO: 7 - protein, 7 aa, Artificial Sequence
  CD5 #1 CDR2-VL
ATSNLQS

SEQ ID NO: 8 - protein, 9 aa, Artificial Sequence
  CD5 #1 CDR3-VL
QQSYTYPWT

SEQ ID NO: 9 - protein, 107 aa, Artificial Sequence
  CD5 #1 Variable Light Chain
DIQMTQSPSSLSASVGDRVTITCRASQDISSYLNWYQQKPGKAPKLLIYATSNLQSGVPSRFSGSGSGTDFTLTISSLQPEDFATYYCQQSYTYPWTFGQGTKVEIK

SEQ ID NO: 10 - protein, 5 aa, Artificial Sequence
  CD5 #4 CDR1-VH
DYAMS

SEQ ID NO: 11 - protein, 17 aa, Artificial Sequence
  CD5 #4 CDR2-VH
AISQSGGSTYYADSVKG

SEQ ID NO: 12 - protein, 12 aa, Artificial Sequence
  CD5 #4 CDR3-VH
DLASVYGAAFDV

SEQ ID NO: 13 - protein, 121 aa, Artificial Sequence
  CD5 #4 Variable Heavy Chain
EVQLVESGGGLVQPGGSLRLSCAASGFTFSDYAMSWVRQAPGKGLEWVSAISQSGGSTYYADSVKGRFTISRDNSKNTLYLQMNSLRAEDTAVYYCAKDLASVYGAAFDVWGQGTLVTVSS

SEQ ID NO: 14 - protein, 11 aa, Artificial Sequence
  CD5 #4 CDR1-VL
RASQTIASYLN

SEQ ID NO: 15 - protein, 7 aa, Artificial Sequence
  CD5 #4 CDR2-VL
AASTLQS

SEQ ID NO: 16 - protein, 9 aa, Artificial Sequence
  CD5 #4 CDR3-VL
QQSYSFPWT

SEQ ID NO: 17 - protein, 107 aa, Artificial Sequence
  CD5 #4 Variable Light Chain
DIQMTQSPSSLSASVGDRVTITCRASQTIASYLNWYQQKPGKAPKLLIYAASTLQSGVPSRFSGSGSGTDFTLTISSLQPEDFATYYCQQSYSFPWTFGQGTKVEIK

SEQ ID NO: 18 - protein, 5 aa, Artificial Sequence
  CD5 #11 CDR1-VH
SYAMS

SEQ ID NO: 19 - protein, 17 aa, Artificial Sequence
  CD5 #11 CDR2-VH
AISSSGGSKYYADSVKG

SEQ ID NO: 20 - protein, 10 aa, Artificial Sequence
  CD5 #11 CDR3-VH
RSYAGEYFDH

SEQ ID NO: 21 - protein, 119 aa, Artificial Sequence
  CD5 #11 Variable Heavy Chain
EVQLVESGGGLVQPGGSLRLSCAASGFTFSSYAMSWVRQAPGKGLEWVSAISSSGGSKYYADSVKGRFTISRDNSKNTLYLQMNSLRAEDTAVYYCAKRSYAGEYFDHWGQGTLVTVSS

SEQ ID NO: 22 - protein, 11 aa, Artificial Sequence
  CD5 #11 CDR1-VL
RASQSISNWLN

SEQ ID NO: 23 - protein, 7 aa, Artificial Sequence
  CD5 #11 CDR2-VL
DASSLQS

SEQ ID NO: 24 - protein, 9 aa, Artificial Sequence
  CD5 #11 CDR3-VL
QQSYSFPWT

SEQ ID NO: 25 - protein, 107 aa, Artificial Sequence
  CD5 #11 Variable Light Chain
DIQMTQSPSSLSASVGDRVTITCRASQSISNWLNWYQQKPGKAPKLLIYDASSLQSGVPSRFSGSGSGTDFTLTISSLQPEDFATYYCQQSYSFPWTFGQGTKVEIK

SEQ ID NO: 26 - protein, 5 aa, Artificial Sequence
  CD5 #14 CDR1-VH
DYAMH

SEQ ID NO: 27 - protein, 17 aa, Artificial Sequence
  CD5 #14 CDR2-VH
AISSSGSYTYYADSVKG

SEQ ID NO: 28 - protein, 10 aa, Artificial Sequence
  CD5 #14 CDR3-VH
GSYYGYYFDI

SEQ ID NO: 29 - protein, 119 aa, Artificial Sequence
  CD5 #14 Variable Heavy Chain
EVQLVESGGGLVQPGGSLRLSCAASGFTFSDYAMHWVRQAPGKGLEWVSAISSSGSYTYYADSVKGRFTISRDNSKNTLYLQMNSLRAEDTAVYYCAKGSYYGYYFDIWGQGTLVTVSS

SEQ ID NO: 30 - protein, 11 aa, Artificial Sequence
  CD5 #14 CDR1-VL
RASQSISNDLN

SEQ ID NO: 31 - protein, 7 aa, Artificial Sequence
  CD5 #14 CDR2-VL
DTSRLQS

SEQ ID NO: 32 - protein, 9 aa, Artificial Sequence
  CD5 #14 CDR3-VL
QQSYSFPWT

SEQ ID NO: 33 - protein, 107 aa, Artificial Sequence
  CD5 #14 Variable Light Chain
DIQMTQSPSSLSASVGDRVTITCRASQSISNDLNWYQQKPGKAPKLLIYDTSRLQSGVPSRFSGSGSGTDFTLTISSLQPEDFATYYCQQSYSFPWTFGQGTKVEIK

SEQ ID NO: 34 - protein, 15 aa, Artificial Sequence
  Linker
GGGGSGGGGSGGGGS

SEQ ID NO: 35 - protein, 289 aa, Artificial Sequence
  CD5 #1 scFv
MKYLLPTAAAGLLLLAAQPAMAEVQLVESGGGLVQPGGSLRLSCAASGFTFSDYGMHWVRQAPGKGLEWVSAISGSGSSTHYADSVKGRFTISRDNSKNTLYLQMNSLRAEDTAVYYCAKGSSSVYSEAMDLWGQGTLVTVSSGGGGSGGGGSGGGGSDIQMTQSPSSLSASVGDRVTITCRASQDISSYLNWYQQKPGKAPKLLIYATSNLQSGVPSRFSGSGSGTDFTLTISSLQPEDFATYYCQQSYTYPWTFGQGTKVEIKASTGPGGQHHHHHHGAWSHPQFEK

SEQ ID NO: 36 - protein, 289 aa, Artificial Sequence
  CD5 #4 scFv
MKYLLPTAAAGLLLLAAQPAMAEVQLVESGGGLVQPGGSLRLSCAASGFTFSDYAMSWVRQAPGKGLEWVSAISQSGGSTYYADSVKGRFTISRDNSKNTLYLQMNSLRAEDTAVYYCAKDLASVYGAAFDVWGQGTLVTVSSGGGGSGGGGSGGGGSDIQMTQSPSSLSASVGDRVTITCRASQTIASYLNWYQQKPGKAPKLLIYAASTLQSGVPSRFSGSGSGTDFTLTISSLQPEDFATYYCQQSYSFPWTFGQGTKVEIKASTGPGGQHHHHHHGAWSHPQFEK

SEQ ID NO: 37 - protein, 287 aa, Artificial Sequence
  CD5 #11 scFv
MKYLLPTAAAGLLLLAAQPAMAEVQLVESGGGLVQPGGSLRLSCAASGFTFSSYAMSWVRQAPGKGLEWVSAISSSGGSKYYADSVKGRFTISRDNSKNTLYLQMNSLRAEDTAVYYCAKRSYAGEYFDHWGQGTLVTVSSGGGGSGGGGSGGGGSDIQMTQSPSSLSASVGDRVTITCRASQSISNWLNWYQQKPGKAPKLLIYDASSLQSGVPSRFSGSGSGTDFTLTISSLQPEDFATYYCQQSYSFPWTFGQGTKVEIKASTGPGGQHHHHHHGAWSHPQFEK

SEQ ID NO: 38 - protein, 287 aa, Artificial Sequence
  CD5 #14 scFv
MKYLLPTAAAGLLLLAAQPAMAEVQLVESGGGLVQPGGSLRLSCAASGFTFSDYAMHWVRQAPGKGLEWVSAISSSGSYTYYADSVKGRFTISRDNSKNTLYLQMNSLRAEDTAVYYCAKGSYYGYYFDIWGQGTLVTVSSGGGGSGGGGSGGGGSDIQMTQSPSSLSASVGDRVTITCRASQSISNDLNWYQQKPGKAPKLLIYDTSRLQSGVPSRFSGSGSGTDFTLTISSLQPEDFATYYCQQSYSFPWTFGQGTKVEIKASTGPGGQHHHHHHGAWSHPQFEK

SEQ ID NO: 39 - protein, 586 aa, Artificial Sequence
  CD5 #1 CAR
MALPVTALLLPLALLLHAARPAAQPAMAEVQLVESGGGLVQPGGSLRLSCAASGFTFSDYGMHWVRQAPGKGLEWVSAISGSGSSTHYADSVKGRFTISRDNSKNTLYLQMNSLRAEDTAVYYCAKGSSSVYSEAMDLWGQGTLVTVSSGGGGSGGGGSGGGGSDIQMTQSPSSLSASVGDRVTITCRASQDISSYLNWYQQKPGKAPKLLIYATSNLQSGVPSRFSGSGSGTDFTLTISSLQPEDFATYYCQQSYTYPWTFGQGTKVEIKASTGPGGREQKLISEEDLKLGVTVSSALSNSIMYFSHFVPVFLPAKPTTTPAPRPPTPAPTIASQPLSLRPEACRPAAGGAVHTRGLDKLVKGKHLCPSPLFPGPSKPFWVLVVVGGVLACYSLLVTVAFIIFWVRSKRSRLLHSDYMNMTPRRPGPTRKHYQPYAPPRDFAAYEFLCARPRRSPAQEDGKVYINMPGRGAAARVKFSRSADAPAYQQGQNQLYNELNLGRREEYDVLDKRRGRDPEMGGKPRRKNPQEGLYNELQKDKMAEAYSEIGMKGERRRGKGHDGLYQGLSTATKDTYDALHMQALPPR

SEQ ID NO: 40 - protein, 586 aa, Artificial Sequence
  CD5 #4 CAR
MALPVTALLLPLALLLHAARPAAQPAMAEVQLVESGGGLVQPGGSLRLSCAASGFTFSDYAMSWVRQAPGKGLEWVSAISQSGGSTYYADSVKGRFTISRDNSKNTLYLQMNSLRAEDTAVYYCAKDLASVYGAAFDVWGQGTLVTVSSGGGGSGGGGSGGGGSDIQMTQSPSSLSASVGDRVTITCRASQTIASYLNWYQQKPGKAPKLLIYAASTLQSGVPSRFSGSGSGTDFTLTISSLQPEDFATYYCQQSYSFPWTFGQGTKVEIKASTGPGGREQKLISEEDLKLGVTVSSALSNSIMYFSHFVPVFLPAKPTTTPAPRPPTPAPTIASQPLSLRPEACRPAAGGAVHTRGLDKLVKGKHLCPSPLFPGPSKPFWVLVVVGGVLACYSLLVTVAFIIFWVRSKRSRLLHSDYMNMTPRRPGPTRKHYQPYAPPRDFAAYEFLCARPRRSPAQEDGKVYINMPGRGAAARVKFSRSADAPAYQQGQNQLYNELNLGRREEYDVLDKRRGRDPEMGGKPRRKNPQEGLYNELQKDKMAEAYSEIGMKGERRRGKGHDGLYQGLSTATKDTYDALHMQALPPR

SEQ ID NO: 41 - protein, 584 aa, Artificial Sequence
  CD5 #11 CAR
MALPVTALLLPLALLLHAARPAAQPAMAEVQLVESGGGLVQPGGSLRLSCAASGFTFSSYAMSWVRQAPGKGLEWVSAISSSGGSKYYADSVKGRFTISRDNSKNTLYLQMNSLRAEDTAVYYCAKRSYAGEYFDHWGQGTLVTVSSGGGGSGGGGSGGGGSDIQMTQSPSSLSASVGDRVTITCRASQSISNWLNWYQQKPGKAPKLLIYDASSLQSGVPSRFSGSGSGTDFTLTISSLQPEDFATYYCQQSYSFPWTFGQGTKVEIKASTGPGGREQKLISEEDLKLGVTVSSALSNSIMYFSHFVPVFLPAKPTTTPAPRPPTPAPTIASQPLSLRPEACRPAAGGAVHTRGLDKLVKGKHLCPSPLFPGPSKPFWVLVVVGGVLACYSLLVTVAFIIFWVRSKRSRLLHSDYMNMTPRRPGPTRKHYQPYAPPRDFAAYEFLCARPRRSPAQEDGKVYINMPGRGAAARVKFSRSADAPAYQQGQNQLYNELNLGRREEYDVLDKRRGRDPEMGGKPRRKNPQEGLYNELQKDKMAEAYSEIGMKGERRRGKGHDGLYQGLSTATKDTYDALHMQALPPR

SEQ ID NO: 42 - protein, 584 aa, Artificial Sequence
  CD5 #14 CAR
MALPVTALLLPLALLLHAARPAAQPAMAEVQLVESGGGLVQPGGSLRLSCAASGFTFSDYAMHWVRQAPGKGLEWVSAISSSGSYTYYADSVKGRFTISRDNSKNTLYLQMNSLRAEDTAVYYCAKGSYYGYYFDIWGQGTLVTVSSGGGGSGGGGSGGGGSDIQMTQSPSSLSASVGDRVTITCRASQSISNDLNWYQQKPGKAPKLLIYDTSRLQSGVPSRFSGSGSGTDFTLTISSLQPEDFATYYCQQSYSFPWTFGQGTKVEIKASTGPGGREQKLISEEDLKLGVTVSSALSNSIMYFSHFVPVFLPAKPTTTPAPRPPTPAPTIASQPLSLRPEACRPAAGGAVHTRGLDKLVKGKHLCPSPLFPGPSKPFWVLVVVGGVLACYSLLVTVAFIIFWVRSKRSRLLHSDYMNMTPRRPGPTRKHYQPYAPPRDFAAYEFLCARPRRSPAQEDGKVYINMPGRGAAARVKFSRSADAPAYQQGQNQLYNELNLGRREEYDVLDKRRGRDPEMGGKPRRKNPQEGLYNELQKDKMAEAYSEIGMKGERRRGKGHDGLYQGLSTATKDTYDALHMQALPPR

SEQ ID NO: 43 - DNA, 68 bp, Artificial Sequence
  Signal peptide
accatggccttaccagtgaccgccttgctcctgccgctggccttactgctccacgccgccaggccggc

SEQ ID NO: 44 - DNA, 32 bp, Artificial Sequence
  Myc
gcgaacaaaaactcatctcagaagaggatctg

SEQ ID NO: 45 - DNA, 204 bp, Artificial Sequence
  Hinge
ggggtcaccgtctcttcagcgctgagcaactccatcatgtacttcagccacttcgtgccggtcttcctgccagcgaagcccaccacgacgccagcgccgcgaccaccaacaccggcgcccaccatcgcgtcgcagcccctgtccctgcgcccagaggcatgccggccagcggcggggggcgcagtgcacacgagggggctggat

SEQ ID NO: 46 - DNA, 252 bp, Artificial Sequence
  Transmembrane
gtgaaagggaaacacctttgtccaagtcccctatttcccggaccttctaagcccttttgggtgctggtggtggttggtggagtcctggcttgctatagcttgctagtaacagtggcctttattattttctgggtgaggagtaagaggagcaggctcctgcacagtgactacatgaacatgactccccgccgccccgggcccacccgcaagcattaccagccctatgccccaccacgcgacttcgcagcctat

SEQ ID NO: 47 - DNA, 72 bp, Artificial Sequence
  DAP10
ctgtgcgcacgcccacgccgcagccccgcccaagaagatggcaaagtctacatcaacatgccaggcaggggc

SEQ ID NO: 48 - DNA, 340 bp, Artificial Sequence
  CD3z
tagagtgaagttcagcaggagcgcagacgcccccgcgtaccagcagggccagaaccagctctataacgagctcaatctaggacgaagagaggagtacgatgttttggacaagagacgtggccgggaccctgagatggggggaaagccgagaaggaagaaccctcaggaaggcctgtacaatgaactgcagaaagataagatggcggaggcctacagtgagattgggatgaaaggcgagcgccggaggggcaaggggcacgatggcctttaccagggtctcagtacagccaccaaggacacctacgacgcccttcacatgcaggccctgccccctcgctaa